European Patent Application EP 4 296 672 A1, published December 27, 2023. Title: Labeled polypeptides, modified polypeptides, methods of producing the polypeptides, reagents containing the polypeptides, and methods of measuring target substance. Applicant: Sysmex Corporation. The sequence listing filed with the application follows.

SEQUENCE LISTING (15 sequences)

SEQ ID NO: 1 - protein, 9 aa, synthetic construct
  REGION 1..9: note = peptide tag
GVLNLAQSP

SEQ ID NO: 2 - protein, 6 aa, synthetic construct
  REGION 1..6: note = peptide tag
GLLQGP

SEQ ID NO: 3 - protein, 5 aa, synthetic construct
  REGION 1..5: note = peptide tag
LLQGP

SEQ ID NO: 4 - protein, 106 aa, synthetic construct
  REGION 1..106: note = light chain of chimeric antibody against p24
TVAAPSVFIFPPSDEQLKSGTASVVCLLNNFYPREAKVQWKVDNALQSGNSQESVTEQDSKDSTYSLSSTLTLSKADYEKHKVYACEVTHQGLSSPVTKSFNRGEC

SEQ ID NO: 5 - DNA, 318 bp, synthetic construct
  misc_feature 1..318: note = light chain of chimeric antibody against p24
  source 1..318: mol_type = other DNA
accgtcgcggcgccgtcggtctttatcttcccgccgagcgatgaacaactgaaatctggtaccgcgagtgtggtttgtctgctgaacaatttttatccgcgtgaagcgaaagtccagtggaaggtggacaacgccctgcagtctggcaatagtcaagaatccgtgaccgaacaagattcaaaagactcgacgtacagcctgagttccaccctgacgctgagcaaggcagattatgaaaaacataaggtgtacgcttgcgaagttacccaccagggtctgtccagtccggttacgaaatcattcaaccgcggcgaatgt

SEQ ID NO: 6 - protein, 112 aa, synthetic construct
  REGION 1..112: note = heavy chain of chimeric antibody against p24
ASTKGPSVFPLAPSSKSTSGGTAALGCLVKDYFPEPVTVSWNSGALTSGVHTFPAVLQSSGLYSLSSVVTVPSSSLGTQTYICNVNHKPSNTKVDKKVEPKSCGVLNLAQSP

SEQ ID NO: 7 - DNA, 336 bp, synthetic construct
  misc_feature 1..336: note = heavy chain of chimeric antibody against p24
  source 1..336: mol_type = other DNA
gctagcacaaaagggcccagcgtgtttccactggctccaagctccaaatctacttctgggggcaccgccgcactgggctgtctggtcaaggactacttcccagagcccgtcaccgtgtcatggaactccggcgcactgacttccggagtccacacctttccagccgtgctgcagtccagcggactgtacagcctgtctagtgtggtcacagtgccttcatccagcctgggaactcagacctatatctgcaacgtgaatcacaagccatcaaatactaaagtcgacaagaaagtggaacccaagagctgtggcgtccttaacctcgcacaaagtcca

SEQ ID NO: 8 - protein, 105 aa, Mus musculus
QPKSSPSVTLFPPSSEELETNKATLVCTITDFYPGVVTVDWKVDGTPVTQGMETTQPSKQSNNKYMASSYLTLTARAWERHSSYSCQVTHEGHTVEKSLSRADCS

SEQ ID NO: 9 - DNA, 315 bp, Mus musculus
  source 1..315: mol_type = genomic DNA
cagcccaagtcttcgccatcagtcaccctgtttccaccttcctctgaagagctcgagactaacaaggccacactggtgtgtacgatcactgatttctacccaggtgtggtgacagtggactggaaggtagatggtacccctgtcactcagggtatggagacaacccagccttccaaacagagcaacaacaagtacatggctagcagctacctgaccctgacagcaagagcatgggaaaggcatagcagttacagctgccaggtcactcatgaaggtcacactgtggagaagagtttgtcccgtgctgactgttcc

SEQ ID NO: 10 - protein, 108 aa, synthetic construct
  REGION 1..108: note = heavy chain of antibody against HBs antigen with peptide tag
AKTTPPSVYPLAPGSAAQTNSMVTLGCLVKGYFPEPVTVTWNSGSLSSGVHTFPAVLQSDLYTLSSSVTVPSSTWPSETVTCNVAHPASSTKVDKKIVPRDCGLLQGP

SEQ ID NO: 11 - DNA, 330 bp, synthetic construct
  misc_feature 1..330: note = heavy chain of antibody against HBs antigen with peptide tag
  source 1..330: mol_type = other DNA
gccaaaacgacacccccatctgtctatccactggcccctggatctgctgcccaaactaactccatggtgaccctgggatgcctggtcaagggctatttccctgagccagtgacagtgacctggaactctggatccctgtccagcggtgtgcacaccttcccagctgtcctgcagtctgacctctacactctgagcagctcagtgactgtcccctccagcacctggcccagcgagaccgtcacctgcaacgttgcccacccggccagcagcaccaaggtggacaagaaaattgtgcccagggattgtggcctgctccagggcccctgataa

SEQ ID NO: 12 - protein, 213 aa, Homo sapiens
QIVLSQSPAILSASPGEKVTMTCRASSSVSYIHWFQQKPGSSPKPWIYATSNLASGVPVRFSGSGSGTSYSLTISRVEAEDAATYYCQQWTSNPPTFGGGTKLEIKRTVAAPSVFIFPPSDEQLKSGTASVVCLLNNFYPREAKVQWKVDNALQSGNSQESVTEQDSKDSTYSLSSTLTLSKADYEKHKVYACEVTHQGLSSPVTKSFNRGEC

SEQ ID NO: 13 - DNA, 636 bp, Homo sapiens
  source 1..636: mol_type = genomic DNA
caaatcgtgcttagccagtcaccagcgatattgtccgctagtcctggagagaaggtgaccatgacctgtagggcatcttccagcgtttcctacattcactggtttcagcagaagccagggtccagccctaaaccctggatctatgccaccagtaaccttgcctcaggggtacctgtgcgattcagcggaagcggtagtggcacctcatactccctgaccattagccgcgttgaagctgaagatgcggctacctactactgccaacagtggacgtctaacccacccacatttggtggcggcactaaactggagatcaagcggactgtggctgcaccatccgtattcatctttccgccctctgatgagcagctgaaatctggcacagctagcgtcgtgtgcctgctgaacaacttctaccctagagaggcaaaagtgcagtggaaggtcgacaatgccctgcagtctggcaattcacaggaatcagtcaccgaacaggactctaaggatagcacgtactccttgagcagcacactcactctctctaaagccgactatgagaagcacaaggtctatgcctgtgaggtgactcatcaagggctgagtagtcccgtcacaaagtccttcaatcgtggagaa

SEQ ID NO: 14 - protein, 234 aa, synthetic construct
  REGION 1..234: note = heavy chain of antibody against CD20 with peptide tag
QVQLQQPGAELVKPGASVKMSCKASGYTFTSYNMHWVKQTPGRGLEWIGAIYPGNGDTSYNQKFKGKATLTADKSSSTAYMQLSSLTSEDSAVYYCARSTYYGGDWYFNVWGAGTTVTVSAASTKGPSVFPLAPSSKSTSGGTAALGCLVKDYFPEPVTVSWNSGALTSGVHTFPAVLQSSGLYSLSSVVTVPSSSLGTQTYICNVNHKPSNTKVDKKAEPKSCDKTHTGLLQG

SEQ ID NO: 15 - DNA, 699 bp, synthetic construct
  misc_feature 1..699: note = heavy chain of antibody against CD20 with peptide tag
  source 1..699: mol_type = other DNA
caggtgcagttgcagcaacctggggcagaactcgtgaagcctggggcatccgttaagatgtcctgtaaagcaagcggctatactttcacttcctacaacatgcattgggtgaaacagactcctggcagaggcttggagtggataggagccatctacccagggaatggtgacacatcttacaaccagaagttcaagggcaaagccaccctcactgccgacaaaagtagctctacagcctatatgcagctgtcatccctgacgagcgaggattcagccgtgtattattgcgctaggtctacctactatggaggcgattggtacttcaatgtgtggggtgccggaactaccgtgactgtgtctgctgcgagcaccaagggtccaagtgtctttccccttgcaccgtccagcaaatccacaagcggaggtactgctgctcttggctgtctggtgaaggactattttccagagccagtgacggttagctggaattcaggcgcccttacatctggggtacacacgtttcctgccgttctgcaaagctcaggactgtacagcctgtctagtgtggtcacagtcccctcaagcagtctcggcacccagacatacatctgcaatgtcaaccacaaaccctccaacaccaaggtcgacaagaaggcagaacccaaaagttgcgataagacccatacagggctgctccaa